European Patent Application EP 4 435 008 A2, published September 25, 2024. Title: Binding Agents. Applicant: UltraHuman Four Limited. Application EP Divisional of European patent application no. 18759711.7, filed August 17, 2018. The sequence listing filed with the application follows.

SEQUENCE LISTING (301 sequences)

SEQ ID NO: 1 - protein, 10 aa, synthetic construct
  REGION 1..10: note = Modified CDR
  VARIANT 3: note = T or any amino acid (for example, S, N or R)
  VARIANT 5: note = T or a conservative substitution of T
  VARIANT 6: note = N or a conservative substitution of N
  VARIANT 9: note = I or a conservative substitution of I
  VARIANT 10: note = F or any amino acid (for example, V or G)
GYXFXXYYXX

SEQ ID NO: 2 - protein, 19 aa, synthetic construct
  REGION 1..19: note = Modified CDR
  VARIANT 1: note = M or a conservative substitution of M
  VARIANT 3: note = I or any amino acid (for example, N, V or D)
  VARIANT 5: note = N or any amino acid (for example, Y)
  VARIANT 7: note = V or any amino acid (for example, G or F)
  VARIANT 8: note = D or a conservative substitution of D
  VARIANT 9: note = G or a conservative substitution of G
  VARIANT 12: note = N or a conservative substitution of N (for example, R)
  VARIANT 13: note = Y or a conservative substitution of Y
  VARIANT 14: note = N or a conservative substitution of N (for example, S)
XGXIXPXXXDTXXXPSFQG

SEQ ID NO: 3 - skipped

SEQ ID NO: 4 - protein, 10 aa, unidentified
  source 1..10: note = Muridae
GYTFTNYYVF

SEQ ID NO: 5 - protein, 7 aa, unidentified
  source 1..7: note = Muridae
GGYTMDY

SEQ ID NO: 6 - protein, 16 aa, synthetic construct
  REGION 1..16: note = Modified CDR
  VARIANT 4: note = Q or a conservative substitution of Q
  VARIANT 6: note = L or a conservative substitution of L
  VARIANT 7: note = L or a conservative substitution of L
  VARIANT 10: note = N or any amino acid (for example, Q, S, T, A or G) or a conservative substitution of N (for example, Q, S, T or G)
  VARIANT 11: note = G or a conservative substitution of G (for example, A)
  VARIANT 12: note = Y or any amino acid (for example, N or S)
  VARIANT 13: note = T or a conservative substitution of T (for example, N)
  VARIANT 16: note = H or any amino acid (for example, D)
RSSXSXXHSXXXXYLX

SEQ ID NO: 7-8 - skipped (2 entries)

SEQ ID NO: 9 - protein, 16 aa, unidentified
  source 1..16: note = Muridae
RSSQSLVHSNGNTYLH

SEQ ID NO: 10 - protein, 7 aa, unidentified
  source 1..7: note = Muridae
KVSYRFS

SEQ ID NO: 11 - protein, 9 aa, unidentified
  source 1..9: note = Muridae
SQNTHVPRT

SEQ ID NO: 12 - protein, 10 aa, synthetic construct
  REGION 1..10: note = Modified CDR
  VARIANT 5: note = T or any amino acid (for example, S, N or R)
  VARIANT 7: note = T or a conservative substitution of T
  VARIANT 8: note = N or a conservative substitution of N
GSGYXFXXYY

SEQ ID NO: 13 - protein, 16 aa, synthetic construct
  REGION 1..16: note = Modified CDR
  VARIANT 2: note = N or any amino acid (for example, Y)
  VARIANT 4: note = V or any amino acid (for example, G or F)
  VARIANT 5: note = D or a conservative substitution of D
  VARIANT 6: note = G or a conservative substitution of G
  VARIANT 9: note = N or a conservative substitution of N (for example, R)
  VARIANT 10: note = Y or a conservative substitution of Y
  VARIANT 11: note = N or a conservative substitution of N (for example, S)
IXPXXXDTXXXPSFQG

SEQ ID NO: 14 - skipped

SEQ ID NO: 15 - protein, 10 aa, unidentified
  source 1..10: note = Muridae
GSGYTFTNYY

SEQ ID NO: 16 - protein, 6 aa, unidentified
  source 1..6: note = Muridae
GGYTMD

SEQ ID NO: 17 - protein, 13 aa, synthetic construct
  REGION 1..13: note = Modified CDR
  VARIANT 3: note = Q or a conservative substitution of Q
  VARIANT 5: note = L or a conservative substitution of L
  VARIANT 6: note = L or a conservative substitution of L
  VARIANT 9: note = N or any amino acid (for example, Q, S, T, A or G) or a conservative substitution of N (for example, Q, S, T or G)
  VARIANT 10: note = G or a conservative substitution of G (for example, A)
  VARIANT 11: note = Y or any amino acid (for example, N or S)
  VARIANT 12: note = T or a conservative substitution of T (for example, N)
SSXSXXHSXXXXY

SEQ ID NO: 18 - skipped

SEQ ID NO: 19 - protein, 13 aa, unidentified
  source 1..13: note = Muridae
SSQSLVHSNGNTY

SEQ ID NO: 20 - protein, 6 aa, unidentified
  source 1..6: note = Muridae
NTHVPR

SEQ ID NO: 21 - protein, 10 aa, synthetic construct
  REGION 1..10: note = Modified CDR
  VARIANT 3: note = T/S/N/R
  VARIANT 5: note = T/N
  VARIANT 6: note = N/S
  VARIANT 9: note = I/V
  VARIANT 10: note = F/V/G
GYXFXXYYXX

SEQ ID NO: 22 - protein, 19 aa, synthetic construct
  REGION 1..19: note = Modified CDR
  VARIANT 1: note = M/I
  VARIANT 3: note = V/N/I/D
  VARIANT 5: note = N/Y
  VARIANT 7: note = V/G/F
  VARIANT 8: note = N/D
  VARIANT 9: note = G/S
  VARIANT 12: note = N/R/K
  VARIANT 13: note = F/Y
  VARIANT 14: note = N/S
XGXIXPXXXDTXXXPSFQG

SEQ ID NO: 23 - skipped

SEQ ID NO: 24 - protein, 10 aa, synthetic construct
  REGION 1..10: note = Modified CDR
  VARIANT 5: note = T/S/N/R
  VARIANT 7: note = T/N
  VARIANT 8: note = N/S
GSGYXFXXYY

SEQ ID NO: 25 - protein, 16 aa, synthetic construct
  REGION 1..16: note = Modified CDR
  VARIANT 2: note = N/Y
  VARIANT 4: note = V/G/F
  VARIANT 5: note = N/D
  VARIANT 6: note = G/S
  VARIANT 9: note = N/R/K
  VARIANT 10: note = F/Y
  VARIANT 11: note = N/S
IXPXXXDTXXXPSFQG

SEQ ID NO: 26 - skipped

SEQ ID NO: 27 - protein, 10 aa, synthetic construct
  REGION 1..10: note = Modified CDR
  VARIANT 3: note = T/S
GYXFTNYYIF

SEQ ID NO: 28 - protein, 19 aa, synthetic construct
  REGION 1..19: note = Modified CDR
  VARIANT 1: note = M/I
  VARIANT 3: note = I/D
  VARIANT 8: note = N/D
  VARIANT 12: note = N/R
  VARIANT 13: note = F/Y
  VARIANT 14: note = N/S
XGXINPVXGDTXXXPSFQG

SEQ ID NO: 29 - protein, 7 aa, synthetic construct
  REGION 1..7: note = Modified CDR
  VARIANT 3: note = F/Y
  VARIANT 5: note = M/P
  VARIANT 7: note = Y/R/K/I
GGXTXDX

SEQ ID NO: 30 - protein, 10 aa, synthetic construct
  REGION 1..10: note = Modified CDR
  VARIANT 5: note = T/S
GSGYXFTNYY

SEQ ID NO: 31 - protein, 16 aa, synthetic construct
  REGION 1..16: note = Modified CDR
  VARIANT 5: note = N/D
  VARIANT 9: note = N/R
  VARIANT 10: note = F/Y
  VARIANT 11: note = N/S
INPVXGDTXXXPSFQG

SEQ ID NO: 32 - protein, 6 aa, synthetic construct
  REGION 1..6: note = Modified CDR
  VARIANT 3: note = F/Y
  VARIANT 5: note = M/P
GGXTXD

SEQ ID NO: 33 - protein, 16 aa, synthetic construct
  REGION 1..16: note = Modified CDR
  VARIANT 4: note = Q/H
  VARIANT 6: note = F/L
  VARIANT 7: note = L/V
  VARIANT 10: note = N/Q/A
  VARIANT 11: note = G/A
  VARIANT 12: note = Y/N/S
  VARIANT 13: note = N/T
  VARIANT 16: note = H/D
RSSXSXXHSXXXXYLX

SEQ ID NO: 34-35 - skipped (2 entries)

SEQ ID NO: 36 - protein, 13 aa, synthetic construct
  REGION 1..13: note = Modified CDR
  VARIANT 3: note = Q/H
  VARIANT 5: note = F/L
  VARIANT 6: note = L/V
  VARIANT 9: note = N/Q/A
  VARIANT 10: note = G/A
  VARIANT 11: note = Y/N/S
  VARIANT 12: note = N/T
SSXSXXHSXXXXY

SEQ ID NO: 37 - skipped

SEQ ID NO: 38 - protein, 16 aa, synthetic construct
  REGION 1..16: note = Modified CDR
  VARIANT 7: note = L/V
  VARIANT 10: note = N/Q/A
  VARIANT 12: note = Y/N
  VARIANT 13: note = N/T
  VARIANT 16: note = H/D
RSSQSLXHSXGXXYLX

SEQ ID NO: 39 - skipped

SEQ ID NO: 40 - protein, 9 aa, synthetic construct
  REGION 1..9: note = Modified CDR
  VARIANT 1: note = F/S
  VARIANT 3: note = Q/N/A
  VARIANT 4: note = T/L
  VARIANT 5: note = Q/H
  VARIANT 6: note = T/V
XQXXXXPRT

SEQ ID NO: 41 - protein, 13 aa, synthetic construct
  REGION 1..13: note = Modified CDR
  VARIANT 6: note = L/V
  VARIANT 9: note = N/Q/A
  VARIANT 11: note = Y/N
  VARIANT 12: note = N/T
SSQSLXHSXGXXY

SEQ ID NO: 42 - skipped

SEQ ID NO: 43 - protein, 10 aa, synthetic construct
  REGION 1..10: note = Modified CDR
GYSFTNYYIF

SEQ ID NO: 44 - protein, 19 aa, synthetic construct
  REGION 1..19: note = Modified CDR
MGDINPVNGDTNYSPSFQG

SEQ ID NO: 45 - protein, 7 aa, synthetic construct
  REGION 1..7: note = Modified CDR
GGYTPDY

SEQ ID NO: 46 - protein, 16 aa, synthetic construct
  REGION 1..16: note = Modified CDR
RSSQSLLHSNGYNYLH

SEQ ID NO: 47 - protein, 7 aa, synthetic construct
  REGION 1..7: note = Modified CDR
KGSNRFS

SEQ ID NO: 48 - protein, 9 aa, synthetic construct
  REGION 1..9: note = Modified CDR
SQNLHVPRT

SEQ ID NO: 49 - protein, 10 aa, synthetic construct
  REGION 1..10: note = Modified CDR
GYTFTNYYIF

SEQ ID NO: 50 - protein, 19 aa, synthetic construct
  REGION 1..19: note = Modified CDR
MGIINPVDGDTNYNPSFQG

SEQ ID NO: 51 - protein, 7 aa, synthetic construct
  REGION 1..7: note = Modified CDR
GGYTMDR

SEQ ID NO: 52 - protein, 16 aa, synthetic construct
  REGION 1..16: note = Modified CDR
RSSQSLLHSNGYTYLH

SEQ ID NO: 53 - protein, 7 aa, synthetic construct
  REGION 1..7: note = Modified CDR
KVSNRLS

SEQ ID NO: 54 - protein, 9 aa, synthetic construct
  REGION 1..9: note = Modified CDR
FQNTHTPRT

SEQ ID NO: 55 - protein, 19 aa, synthetic construct
  REGION 1..19: note = Modified CDR
IGDINPVNGDTNFSPSFQG

SEQ ID NO: 56 - protein, 7 aa, synthetic construct
  REGION 1..7: note = Modified CDR
GGYTMDK

SEQ ID NO: 57 - protein, 16 aa, synthetic construct
  REGION 1..16: note = Modified CDR
RSSQSLVHSNGYTYLH

SEQ ID NO: 58 - protein, 7 aa, synthetic construct
  REGION 1..7: note = Modified CDR
KGSYRAS

SEQ ID NO: 59 - protein, 9 aa, synthetic construct
  REGION 1..9: note = Modified CDR
SQNTQTPRT

SEQ ID NO: 60 - protein, 19 aa, synthetic construct
  REGION 1..19: note = Modified CDR
MGIINPVNGDTNYNPSFQG

SEQ ID NO: 61 - protein, 7 aa, synthetic construct
  REGION 1..7: note = Modified CDR
GGYTMGK

SEQ ID NO: 62 - protein, 16 aa, synthetic construct
  REGION 1..16: note = Modified CDR
RSSQSLVHSNGNTYLD

SEQ ID NO: 63 - protein, 7 aa, synthetic construct
  REGION 1..7: note = Modified CDR
KGSYRFS

SEQ ID NO: 64 - protein, 9 aa, synthetic construct
  REGION 1..9: note = Modified CDR
SQATHTPRT

SEQ ID NO: 65 - protein, 19 aa, synthetic construct
  REGION 1..19: note = Modified CDR
MGIINPVDGDTRYSPSFQG

SEQ ID NO: 66 - protein, 7 aa, synthetic construct
  REGION 1..7: note = Modified CDR
GGFTMDY

SEQ ID NO: 67 - protein, 7 aa, synthetic construct
  REGION 1..7: note = Modified CDR
KGSNRAS

SEQ ID NO: 68 - protein, 9 aa, synthetic construct
  REGION 1..9: note = Modified CDR
SQNTHTPRT

SEQ ID NO: 69 - protein, 19 aa, synthetic construct
  REGION 1..19: note = Modified CDR
IGIINPVDGDTRYSPSFQG

SEQ ID NO: 70 - protein, 7 aa, synthetic construct
  REGION 1..7: note = Modified CDR
GGYTMDI

SEQ ID NO: 71 - protein, 7 aa, synthetic construct
  REGION 1..7: note = Modified CDR
LGSNRFS

SEQ ID NO: 72 - protein, 7 aa, synthetic construct
  REGION 1..7: note = Modified CDR
LGSNRAS

SEQ ID NO: 73 - protein, 9 aa, synthetic construct
  REGION 1..9: note = Modified CDR
SQATQTPRT

SEQ ID NO: 74 - protein, 19 aa, synthetic construct
  REGION 1..19: note = Modified CDR
MGIINPVDGDTRYNPSFQG

SEQ ID NO: 75 - protein, 7 aa, synthetic construct
  REGION 1..7: note = Modified CDR
KGSNRLS

SEQ ID NO: 76 - protein, 9 aa, synthetic construct
  REGION 1..9: note = Modified CDR
FQNTQTPRT

SEQ ID NO: 77 - protein, 7 aa, synthetic construct
  REGION 1..7: note = Modified CDR
LGSNRLS

SEQ ID NO: 78 - protein, 16 aa, synthetic construct
  REGION 1..16: note = Modified CDR
RSSQSLLHSQGYTYLH

SEQ ID NO: 79 - protein, 9 aa, synthetic construct
  REGION 1..9: note = Modified CDR
FQQTHTPRT

SEQ ID NO: 80 - protein, 16 aa, synthetic construct
  REGION 1..16: note = Modified CDR
RSSQSLLHSSGYNYLH

SEQ ID NO: 81 - protein, 16 aa, synthetic construct
  REGION 1..16: note = Modified CDR
RSSQSLLHSGGYNYLH

SEQ ID NO: 82 - protein, 16 aa, synthetic construct
  REGION 1..16: note = Modified CDR
RSSQSLLHSAGYNYLH

SEQ ID NO: 83 - protein, 16 aa, synthetic construct
  REGION 1..16: note = Modified CDR
RSSQSLLHSTGYNYLH

SEQ ID NO: 84 - protein, 16 aa, synthetic construct
  REGION 1..16: note = Modified CDR
RSSQSLLHSNAYNYLH

SEQ ID NO: 85 - protein, 7 aa, synthetic construct
  REGION 1..7: note = Modified CDR
KVSNRFS

SEQ ID NO: 86 - protein, 10 aa, synthetic construct
  REGION 1..10: note = Modified CDR
GSGYSFTNYY

SEQ ID NO: 87 - protein, 16 aa, synthetic construct
  REGION 1..16: note = Modified CDR
INPVNGDTNYSPSFQG

SEQ ID NO: 88 - protein, 6 aa, synthetic construct
  REGION 1..6: note = Modified CDR
GGYTPD

SEQ ID NO: 89 - protein, 13 aa, synthetic construct
  REGION 1..13: note = Modified CDR
SSQSLLHSNGYNY

SEQ ID NO: 90 - protein, 6 aa, synthetic construct
  REGION 1..6: note = Modified CDR
NLHVPR

SEQ ID NO: 91 - protein, 16 aa, synthetic construct
  REGION 1..16: note = Modified CDR
INPVDGDTNYNPSFQG

SEQ ID NO: 92 - protein, 13 aa, synthetic construct
  REGION 1..13: note = Modified CDR
SSQSLLHSNGYTY

SEQ ID NO: 93 - protein, 6 aa, synthetic construct
  REGION 1..6: note = Modified CDR
NTHTPR

SEQ ID NO: 94 - protein, 16 aa, synthetic construct
  REGION 1..16: note = Modified CDR
INPVNGDTNFSPSFQG

SEQ ID NO: 95 - protein, 13 aa, synthetic construct
  REGION 1..13: note = Modified CDR
SSQSLVHSNGYTY

SEQ ID NO: 96 - protein, 6 aa, synthetic construct
  REGION 1..6: note = Modified CDR
NTQTPR

SEQ ID NO: 97 - protein, 16 aa, synthetic construct
  REGION 1..16: note = Modified CDR
INPVNGDTNYNPSFQG

SEQ ID NO: 98 - protein, 6 aa, synthetic construct
  REGION 1..6: note = Modified CDR
GGYTMG

SEQ ID NO: 99 - protein, 6 aa, synthetic construct
  REGION 1..6: note = Modified CDR
ATHTPR

SEQ ID NO: 100 - protein, 16 aa, synthetic construct
  REGION 1..16: note = Modified CDR
INPVDGDTRYSPSFQG

SEQ ID NO: 101 - protein, 6 aa, synthetic construct
  REGION 1..6: note = Modified CDR
GGFTMD

SEQ ID NO: 102 - protein, 6 aa, synthetic construct
  REGION 1..6: note = Modified CDR
ATQTPR

SEQ ID NO: 103 - protein, 16 aa, synthetic construct
  REGION 1..16: note = Modified CDR
INPVDGDTRYNPSFQG

SEQ ID NO: 104 - protein, 13 aa, synthetic construct
  REGION 1..13: note = Modified CDR
SSQSLLHSQGYTY

SEQ ID NO: 105 - protein, 6 aa, synthetic construct
  REGION 1..6: note = Modified CDR
QTHTPR

SEQ ID NO: 106 - protein, 13 aa, synthetic construct
  REGION 1..13: note = Modified CDR
SSQSLLHSSGYNY

SEQ ID NO: 107 - protein, 13 aa, synthetic construct
  REGION 1..13: note = Modified CDR
SSQSLLHSGGYNY

SEQ ID NO: 108 - protein, 13 aa, synthetic construct
  REGION 1..13: note = Modified CDR
SSQSLLHSAGYNY

SEQ ID NO: 109 - protein, 13 aa, synthetic construct
  REGION 1..13: note = Modified CDR
SSQSLLHSTGYNY

SEQ ID NO: 110 - protein, 13 aa, synthetic construct
  REGION 1..13: note = Modified CDR
SSQSLLHSNAYNY

SEQ ID NO: 111 - protein, 19 aa, synthetic construct
  REGION 1..19: note = Modified CDR
  VARIANT 12: note = N/R
  VARIANT 14: note = N/S
MGIINPVDGDTXYXPSFQG

SEQ ID NO: 112 - protein, 16 aa, synthetic construct
  REGION 1..16: note = Modified CDR
  VARIANT 10: note = N/A
  VARIANT 13: note = N/T
RSSQSLLHSXGYXYLH

SEQ ID NO: 113 - protein, 7 aa, synthetic construct
  REGION 1..7: note = Modified CDR
  VARIANT 6: note = L/F
KVSNRXS

SEQ ID NO: 114 - protein, 16 aa, synthetic construct
  REGION 1..16: note = Modified CDR
  VARIANT 9: note = N/R
  VARIANT 11: note = N/S
INPVDGDTXYXPSFQG

SEQ ID NO: 115 - protein, 13 aa, synthetic construct
  REGION 1..13: note = Modified CDR
  VARIANT 9: note = N/A
  VARIANT 12: note = N/T
SSQSLLHSXGYXY

SEQ ID NO: 116 - protein, 9 aa, unidentified
  source 1..9: note = Muridae
LVHSNGNTY

SEQ ID NO: 117 - protein, 9 aa, unidentified
  source 1..9: note = Muridae
LLIYKVSYR

SEQ ID NO: 118 - protein, 9 aa, unidentified
  source 1..9: note = Muridae
YRFSGVPDR

SEQ ID NO: 119 - protein, 9 aa, unidentified
  source 1..9: note = Muridae
LIYKVSYRF

SEQ ID NO: 120 - protein, 16 aa, unidentified
  source 1..16: note = Muridae
LLIYKVSYRFSGVPDR

SEQ ID NO: 121 - protein, 9 aa, unidentified
  source 1..9: note = Muridae
VGVYYCFQN

SEQ ID NO: 122 - protein, 15 aa, synthetic construct
  REGION 1..15: note = Modified CDR
AGVYYCFQNTHTPRT

SEQ ID NO: 123 - protein, 19 aa, unidentified
  source 1..19: note = Muridae
IGDINPVNGDTNFNEKFKN

SEQ ID NO: 124 - protein, 5 aa, unidentified
  source 1..5: note = Muridae
NYYVF

SEQ ID NO: 125 - protein, 17 aa, unidentified
  source 1..17: note = Muridae
DINPVNGDTNFNEKFKN

SEQ ID NO: 126 - protein, 7 aa, unidentified
  source 1..7: note = Muridae
GYTFTNY

SEQ ID NO: 127 - protein, 6 aa, unidentified
  source 1..6: note = Muridae
NPVNGD

SEQ ID NO: 128 - protein, 8 aa, unidentified
  source 1..8: note = Muridae
GYTFTNYY

SEQ ID NO: 129 - protein, 8 aa, unidentified
  source 1..8: note = Muridae
INPVNGDT

SEQ ID NO: 130 - protein, 9 aa, unidentified
  source 1..9: note = Muridae
TRGGYTMDY

SEQ ID NO: 131 - protein, 11 aa, unidentified
  source 1..11: note = Muridae
QSLVHSNGNTY

SEQ ID NO: 132 - protein, 16 aa, unidentified
  source 1..16: note = Muridae
INPVNGDTNFNEKFKN

SEQ ID NO: 133 - protein, 10 aa, unidentified
  source 1..10: note = Muridae
DINPVNGDTN

SEQ ID NO: 134 - protein, 6 aa, unidentified
  source 1..6: note = Muridae
TNYYVF

SEQ ID NO: 135 - protein, 12 aa, unidentified
  source 1..12: note = Muridae
IGDINPVNGDTN

SEQ ID NO: 136 - protein, 8 aa, unidentified
  source 1..8: note = Muridae
TRGGYTMD

SEQ ID NO: 137 - protein, 11 aa, unidentified
  source 1..11: note = Muridae
HSNGNTYLHWY

SEQ ID NO: 138 - protein, 10 aa, unidentified
  source 1..10: note = Muridae
LLIYKVSYRF

SEQ ID NO: 139 - protein, 8 aa, unidentified
  source 1..8: note = Muridae
SQNTHVPR

SEQ ID NO: 140 - protein, 116 aa, unidentified
  DOMAIN 1..116: note = VH DOMAIN
  source 1..116: note = Muridae
EVQLQQFGAELVKPGASMKLSCKASGYTFTNYYVFWVKQRPGQGLEWIGDINPVNGDTNFNEKFKNKATLTVDKSSTTTYLQLSSLTSEDSAVYYCTRGGYTMDYWGQGTLVTVSS

SEQ ID NO: 141 - protein, 116 aa, synthetic construct
  REGION 1..116: note = VH DOMAIN
EVQLVQSGAEVKKPGESLKISCKGSGYTFTNYYVFWVRQMPGKGLEWIGDINPVNGDTNFNESFQGQVTISADKSISTAYLQWSSLKASDTAMYYCARGGYTMDYWGQGTLVTVSS

SEQ ID NO: 142 - protein, 112 aa, unidentified
  DOMAIN 1..112: note = VL DOMAIN
  source 1..112: note = Muridae
DVVMTQTPLSLSVSLGDQASISCRSSQSLVHSNGNTYLHWYLQKPGQSPKLLIYKVSYRFSGVPDRFSGSGSGTDFTLKISRVEAEDLGVYFCSQNTHVPRTFGQGTKVEIK

SEQ ID NO: 143 - protein, 112 aa, synthetic construct
  REGION 1..112: note = VL DOMAIN
DIVMTQSPLSLPVTPGEPASISCRSSQSLVHSNGNTYLHWYLQKPGQSPQLLIYKVSYRFSGVPDRFSGSGSGTDFTLKISRVEAEDVGVYYCSQNTHVPRTFGQGTKVEIK

SEQ ID NO: 144 - protein, 16 aa, synthetic construct
  REGION 1..16: note = Modified CDR
RSSHSLVHSNGNTYLH

SEQ ID NO: 145 - protein, 10 aa, synthetic construct
  REGION 1..10: note = Modified CDR
GYNFTNYYIF

SEQ ID NO: 146 - protein, 19 aa, synthetic construct
  REGION 1..19: note = Modified CDR
MGDINPFNGDTNFNPSFQG

SEQ ID NO: 147 - protein, 16 aa, synthetic construct
  REGION 1..16: note = Modified CDR
RSSQSFLHSNGNNYLH

SEQ ID NO: 148 - protein, 9 aa, synthetic construct
  REGION 1..9: note = Modified CDR
LQNTHTPRT

SEQ ID NO: 149 - protein, 10 aa, synthetic construct
  REGION 1..10: note = Modified CDR
GYRFTNYYIF

SEQ ID NO: 150 - protein, 19 aa, synthetic construct
  REGION 1..19: note = Modified CDR
MGDINPGDGDTNFNPSFQG

SEQ ID NO: 151 - protein, 7 aa, synthetic construct
  REGION 1..7: note = Modified CDR
GGHTMDY

SEQ ID NO: 152 - protein, 16 aa, synthetic construct
  REGION 1..16: note = Modified CDR
RSSQSLLHSNGNNYLD

SEQ ID NO: 153 - protein, 7 aa, synthetic construct
  REGION 1..7: note = Modified CDR
KGSNRSS

SEQ ID NO: 154 - protein, 9 aa, synthetic construct
  REGION 1..9: note = Modified CDR
MQALHTPWT

SEQ ID NO: 155 - protein, 10 aa, synthetic construct
  REGION 1..10: note = Modified CDR
GYRFTNYYVF

SEQ ID NO: 156 - protein, 19 aa, synthetic construct
  REGION 1..19: note = Modified CDR
MGDINPGNGDTNFNPSFQG

SEQ ID NO: 157 - protein, 7 aa, synthetic construct
  REGION 1..7: note = Modified CDR
GGITMDY

SEQ ID NO: 158 - protein, 16 aa, synthetic construct
  REGION 1..16: note = Modified CDR
RSSQSLLHSNGNNYLH

SEQ ID NO: 159 - protein, 9 aa, synthetic construct
  REGION 1..9: note = Modified CDR
MQALHVPRT

SEQ ID NO: 160 - protein, 10 aa, synthetic construct
  REGION 1..10: note = Modified CDR
GYSFNNYYIF

SEQ ID NO: 161 - protein, 19 aa, synthetic construct
  REGION 1..19: note = Modified CDR
MGDINPGNGDTNYNPSFQG

SEQ ID NO: 162 - protein, 7 aa, synthetic construct
  REGION 1..7: note = Modified CDR
GGQTMDQ

SEQ ID NO: 163 - protein, 16 aa, synthetic construct
  REGION 1..16: note = Modified CDR
RSSQSLLHSNGNTYLD

SEQ ID NO: 164 - protein, 9 aa, synthetic construct
  REGION 1..9: note = Modified CDR
MQALQVPWT

SEQ ID NO: 165 - protein, 19 aa, synthetic construct
  REGION 1..19: note = Modified CDR
MGDINPGNGDTNYSPSFQG

SEQ ID NO: 166 - protein, 7 aa, synthetic construct
  REGION 1..7: note = Modified CDR
GGYIMDY

SEQ ID NO: 167 - protein, 16 aa, synthetic construct
  REGION 1..16: note = Modified CDR
RSSQSLLHSNGNTYLH

SEQ ID NO: 168 - protein, 7 aa, synthetic construct
  REGION 1..7: note = Modified CDR
KGSYRLS

SEQ ID NO: 169 - protein, 9 aa, synthetic construct
  REGION 1..9: note = Modified CDR
MQATHVPWT

SEQ ID NO: 170 - protein, 10 aa, synthetic construct
  REGION 1..10: note = Modified CDR
GYSFTSYYIF

SEQ ID NO: 171 - protein, 19 aa, synthetic construct
  REGION 1..19: note = Modified CDR
MGDINPGNGDTRFNPSFQG

SEQ ID NO: 172 - protein, 7 aa, synthetic construct
  REGION 1..7: note = Modified CDR
GGYTADY

SEQ ID NO: 173 - protein, 16 aa, synthetic construct
  REGION 1..16: note = Modified CDR
RSSQSLLHSNGSNYLH

SEQ ID NO: 174 - protein, 7 aa, synthetic construct
  REGION 1..7: note = Modified CDR
KVSNRAS

SEQ ID NO: 175 - protein, 9 aa, synthetic construct
  REGION 1..9: note = Modified CDR
MQATQVPWT

SEQ ID NO: 176 - protein, 10 aa, synthetic construct
  REGION 1..10: note = Modified CDR
GYSFTSYYIV

SEQ ID NO: 177 - protein, 19 aa, synthetic construct
  REGION 1..19: note = Modified CDR
MGDINPGNGDTRFSPSFQG

SEQ ID NO: 178 - protein, 7 aa, synthetic construct
  REGION 1..7: note = Modified CDR
GGYTLDY

SEQ ID NO: 179 - protein, 9 aa, synthetic construct
  REGION 1..9: note = Modified CDR
MQNLQTPRT

SEQ ID NO: 180 - protein, 10 aa, synthetic construct
  REGION 1..10: note = Modified CDR
GYSFTSYYVF

SEQ ID NO: 181 - protein, 19 aa, synthetic construct
  REGION 1..19: note = Modified CDR
MGDINPGNGDTRYNPSFQG

SEQ ID NO: 182 - protein, 7 aa, synthetic construct
  REGION 1..7: note = Modified CDR
GGYTMDA

SEQ ID NO: 183 - protein, 16 aa, synthetic construct
  REGION 1..16: note = Modified CDR
RSSQSLLHSNGYTYLD

SEQ ID NO: 184 - protein, 9 aa, synthetic construct
  REGION 1..9: note = Modified CDR
MQNTHIPRT

SEQ ID NO: 185 - protein, 10 aa, synthetic construct
  REGION 1..10: note = Modified CDR
GYSFTSYYVG

SEQ ID NO: 186 - protein, 19 aa, synthetic construct
  REGION 1..19: note = Modified CDR
MGDINPGNGDTRYSPSFQG

SEQ ID NO: 187 - protein, 7 aa, synthetic construct
  REGION 1..7: note = Modified CDR
GGYTMDE

SEQ ID NO: 188 - protein, 7 aa, synthetic construct
  REGION 1..7: note = Modified CDR
KVSYRAS

SEQ ID NO: 189 - protein, 9 aa, synthetic construct
  REGION 1..9: note = Modified CDR
MQNTHTLRT

SEQ ID NO: 190 - protein, 19 aa, synthetic construct
  REGION 1..19: note = Modified CDR
MGDINPGNSDTNFNPSFQG

SEQ ID NO: 191 - protein, 7 aa, synthetic construct
  REGION 1..7: note = Modified CDR
GGYTMDF

SEQ ID NO: 192 - protein, 16 aa, synthetic construct
  REGION 1..16: note = Modified CDR
RSSQSLVHSNGNNYLD

SEQ ID NO: 193 - protein, 7 aa, synthetic construct
  REGION 1..7: note = Modified CDR
KVSYRLS

SEQ ID NO: 194 - protein, 9 aa, synthetic construct
  REGION 1..9: note = Modified CDR
MQNTHTPRT

SEQ ID NO: 195 - protein, 10 aa, synthetic construct
  REGION 1..10: note = Modified CDR
GYTFTSYYIF

SEQ ID NO: 196 - protein, 19 aa, synthetic construct
  REGION 1..19: note = Modified CDR
MGDINPGNSDTNYNPSFQG

SEQ ID NO: 197 - protein, 7 aa, synthetic construct
  REGION 1..7: note = Modified CDR
GGYTMDH

SEQ ID NO: 198 - protein, 9 aa, synthetic construct
  REGION 1..9: note = Modified CDR
MQNTHVPRT

SEQ ID NO: 199 - protein, 10 aa, synthetic construct
  REGION 1..10: note = Modified CDR
GYTFTSYYVF

SEQ ID NO: 200 - protein, 19 aa, synthetic construct
  REGION 1..19: note = Modified CDR
MGDINPVDGDTKYNPSFQG

SEQ ID NO: 201 - protein, 16 aa, synthetic construct
  REGION 1..16: note = Modified CDR
RSSQSLVHSNGNNYLH

SEQ ID NO: 202 - protein, 9 aa, synthetic construct
  REGION 1..9: note = Modified CDR
MQNTQTPRT

SEQ ID NO: 203 - protein, 19 aa, synthetic construct
  REGION 1..19: note = Modified CDR
MGDINPVDGDTNFNPSFQG

SEQ ID NO: 204 - protein, 9 aa, synthetic construct
  REGION 1..9: note = Modified CDR
MQTTHTPRT

SEQ ID NO: 205 - protein, 19 aa, synthetic construct
  REGION 1..19: note = Modified CDR
MGDINPVDGDTNFSPSFQG

SEQ ID NO: 206 - protein, 7 aa, synthetic construct
  REGION 1..7: note = Modified CDR
GGYTMDL

SEQ ID NO: 207 - protein, 16 aa, synthetic construct
  REGION 1..16: note = Modified CDR
RSSQSLVHSNGYNYLH

SEQ ID NO: 208 - protein, 7 aa, synthetic construct
  REGION 1..7: note = Modified CDR
LGSYRAS

SEQ ID NO: 209 - protein, 9 aa, synthetic construct
  REGION 1..9: note = Modified CDR
MQTTQIPRT

SEQ ID NO: 210 - protein, 19 aa, synthetic construct
  REGION 1..19: note = Modified CDR
MGDINPVDGDTNYNPSFQG

SEQ ID NO: 211 - protein, 7 aa, synthetic construct
  REGION 1..7: note = Modified CDR
GGYTMDM

SEQ ID NO: 212 - protein, 16 aa, synthetic construct
  REGION 1..16: note = Modified CDR
RSSQSLVHSNGYTYLD

SEQ ID NO: 213 - protein, 7 aa, synthetic construct
  REGION 1..7: note = Modified CDR
LGSYRFS

SEQ ID NO: 214 - protein, 9 aa, synthetic construct
  REGION 1..9: note = Modified CDR
SQATHFPRT

SEQ ID NO: 215 - protein, 19 aa, synthetic construct
  REGION 1..19: note = Modified CDR
MGDINPVDGDTNYSPSFQG

SEQ ID NO: 216 - protein, 7 aa, synthetic construct
  REGION 1..7: note = Modified CDR
GGYTMDN

SEQ ID NO: 217 - protein, 7 aa, synthetic construct
  REGION 1..7: note = Modified CDR
LGSYRLS

SEQ ID NO: 218 - protein, 19 aa, synthetic construct
  REGION 1..19: note = Modified CDR
MGDINPVDGDTRFNPSFQG

SEQ ID NO: 219 - protein, 7 aa, synthetic construct
  REGION 1..7: note = Modified CDR
GGYTMDQ

SEQ ID NO: 220 - protein, 7 aa, synthetic construct
  REGION 1..7: note = Modified CDR
LVSNRAS

SEQ ID NO: 221 - protein, 9 aa, synthetic construct
  REGION 1..9: note = Modified CDR
SQNIQTPRT

SEQ ID NO: 222 - protein, 19 aa, synthetic construct
  REGION 1..19: note = Modified CDR
MGDINPVDGDTRYNPSFQG

SEQ ID NO: 223 - protein, 7 aa, synthetic construct
  REGION 1..7: note = Modified CDR
LVSNRFS

SEQ ID NO: 224 - protein, 9 aa, synthetic construct
  REGION 1..9: note = Modified CDR
SQNLHTPRT

SEQ ID NO: 225 - protein, 19 aa, synthetic construct
  REGION 1..19: note = Modified CDR
MGDINPVDGDTRYSPSFQG

SEQ ID NO: 226 - protein, 7 aa, synthetic construct
  REGION 1..7: note = Modified CDR
GGYTMDT

SEQ ID NO: 227 - protein, 7 aa, synthetic construct
  REGION 1..7: note = Modified CDR
LVSNRLS

SEQ ID NO: 228 - protein, 9 aa, synthetic construct
  REGION 1..9: note = Modified CDR
SQNLQTPRT

SEQ ID NO: 229 - protein, 19 aa, synthetic construct
  REGION 1..19: note = Modified CDR
MGDINPVDSDTKFNPSFQG

SEQ ID NO: 230 - protein, 7 aa, synthetic construct
  REGION 1..7: note = Modified CDR
GGYTMDV

SEQ ID NO: 231 - protein, 7 aa, synthetic construct
  REGION 1..7: note = Modified CDR
LVSYRAS

SEQ ID NO: 232 - protein, 9 aa, synthetic construct
  REGION 1..9: note = Modified CDR
SQNMHTPRT

SEQ ID NO: 233 - protein, 19 aa, synthetic construct
  REGION 1..19: note = Modified CDR
MGDINPVDSDTNFNPSFQG

SEQ ID NO: 234 - protein, 7 aa, synthetic construct
  REGION 1..7: note = Modified CDR
GGYTMDW

SEQ ID NO: 235 - protein, 7 aa, synthetic construct
  REGION 1..7: note = Modified CDR
MGSNRFS

SEQ ID NO: 236 - protein, 9 aa, synthetic construct
  REGION 1..9: note = Modified CDR
SQNTHFPRT

SEQ ID NO: 237 - protein, 19 aa, synthetic construct
  REGION 1..19: note = Modified CDR
MGDINPVDSDTNYNPSFQG

SEQ ID NO: 238 - protein, 7 aa, synthetic construct
  REGION 1..7: note = Modified CDR
MGSYRLS

SEQ ID NO: 239 - protein, 9 aa, synthetic construct
  REGION 1..9: note = Modified CDR
SQNTHVPWT

SEQ ID NO: 240 - protein, 19 aa, synthetic construct
  REGION 1..19: note = Modified CDR
MGDINPVDSDTNYSPSFQG

SEQ ID NO: 241 - protein, 7 aa, synthetic construct
  REGION 1..7: note = Modified CDR
MVSNRFS

SEQ ID NO: 242 - protein, 9 aa, synthetic construct
  REGION 1..9: note = Modified CDR
SQNTQAPRT

SEQ ID NO: 243 - protein, 19 aa, synthetic construct
  REGION 1..19: note = Modified CDR
MGDINPVDSDTRFNPSFQG

SEQ ID NO: 244 - protein, 7 aa, synthetic construct
  REGION 1..7: note = Modified CDR
GGYTRDY

SEQ ID NO: 245 - protein, 19 aa, synthetic construct
  REGION 1..19: note = Modified CDR
MGDINPVDSDTRYNPSFQG

SEQ ID NO: 246 - protein, 7 aa, synthetic construct
  REGION 1..7: note = Modified CDR
GGYTTDS

SEQ ID NO: 247 - protein, 9 aa, synthetic construct
  REGION 1..9: note = Modified CDR
SQNTQTPWT

SEQ ID NO: 248 - protein, 19 aa, synthetic construct
  REGION 1..19: note = Modified CDR
MGDINPVDSDTRYSPSFQG

SEQ ID NO: 249 - protein, 7 aa, synthetic construct
  REGION 1..7: note = Modified CDR
GGYTTDW

SEQ ID NO: 250 - protein, 9 aa, synthetic construct
  REGION 1..9: note = Modified CDR
SQNTQVPRT

SEQ ID NO: 251 - protein, 19 aa, synthetic construct
  REGION 1..19: note = Modified CDR
MGDINPVNGDTKYNPSFQG

SEQ ID NO: 252 - protein, 7 aa, synthetic construct
  REGION 1..7: note = Modified CDR
GGYTTDY

SEQ ID NO: 253 - protein, 9 aa, synthetic construct
  REGION 1..9: note = Modified CDR
SQSTHVPRT

SEQ ID NO: 254 - protein, 19 aa, synthetic construct
  REGION 1..19: note = Modified CDR
MGDINPVNGDTNFSPSFQG

SEQ ID NO: 255 - protein, 7 aa, synthetic construct
  REGION 1..7: note = Modified CDR
GGYVMDY

SEQ ID NO: 256 - protein, 9 aa, synthetic construct
  REGION 1..9: note = Modified CDR
SQTTHIPRT

SEQ ID NO: 257 - protein, 19 aa, synthetic construct
  REGION 1..19: note = Modified CDR
MGDINPVNGDTNYNPSFQG

SEQ ID NO: 258 - protein, 9 aa, synthetic construct
  REGION 1..9: note = Modified CDR
SQTTHVPRT

SEQ ID NO: 259 - protein, 9 aa, synthetic construct
  REGION 1..9: note = Modified CDR
SQTTQTPRT

SEQ ID NO: 260 - protein, 19 aa, synthetic construct
  REGION 1..19: note = Modified CDR
MGDINPVNGDTRFNPSFQG

SEQ ID NO: 261 - protein, 9 aa, synthetic construct
  REGION 1..9: note = Modified CDR
TQNTHTPRT

SEQ ID NO: 262 - protein, 19 aa, synthetic construct
  REGION 1..19: note = Modified CDR
MGDINPVNGDTRFSPSFQG

SEQ ID NO: 263 - protein, 9 aa, synthetic construct
  REGION 1..9: note = Modified CDR
VQNTQVPRT

SEQ ID NO: 264 - protein, 19 aa, synthetic construct
  REGION 1..19: note = Modified CDR
MGDINPVNGDTRYNPSFQG

SEQ ID NO: 265 - protein, 19 aa, synthetic construct
  REGION 1..19: note = Modified CDR
MGDINPVNGDTRYSPSFQG

SEQ ID NO: 266 - protein, 19 aa, synthetic construct
  REGION 1..19: note = Modified CDR
MGDINPVNSDTKYNPSFQG

SEQ ID NO: 267 - protein, 19 aa, synthetic construct
  REGION 1..19: note = Modified CDR
MGDINPVNSDTNFNPSFQG

SEQ ID NO: 268 - protein, 19 aa, synthetic construct
  REGION 1..19: note = Modified CDR
MGDINPVNSDTNYSPSFQG

SEQ ID NO: 269 - protein, 19 aa, synthetic construct
  REGION 1..19: note = Modified CDR
MGDINPVNSDTRFNPSFQG

SEQ ID NO: 270 - protein, 19 aa, synthetic construct
  REGION 1..19: note = Modified CDR
MGDINPVNSDTRFSPSFQG

SEQ ID NO: 271 - protein, 19 aa, synthetic construct
  REGION 1..19: note = Modified CDR
MGDINPVNSDTRYNPSFQG

SEQ ID NO: 272 - protein, 19 aa, synthetic construct
  REGION 1..19: note = Modified CDR
MGDINPVNSDTRYSPSFQG

SEQ ID NO: 273 - protein, 19 aa, synthetic construct
  REGION 1..19: note = Modified CDR
MGDIYPGNSDTKYNPSFQG

SEQ ID NO: 274 - protein, 19 aa, synthetic construct
  REGION 1..19: note = Modified CDR
MGDIYPVNGDTRYNPSFQG

SEQ ID NO: 275 - protein, 19 aa, synthetic construct
  REGION 1..19: note = Modified CDR
MGIINPGNGDTRYNPSFQG

SEQ ID NO: 276 - protein, 19 aa, synthetic construct
  REGION 1..19: note = Modified CDR
MGIINPVDGDTKYNPSFQG

SEQ ID NO: 277 - protein, 19 aa, synthetic construct
  REGION 1..19: note = Modified CDR
MGIINPVDGDTNYSPSFQG

SEQ ID NO: 278 - protein, 19 aa, synthetic construct
  REGION 1..19: note = Modified CDR
MGIINPVDGDTRFNPSFQG

SEQ ID NO: 279 - protein, 19 aa, synthetic construct
  REGION 1..19: note = Modified CDR
MGIINPVDGDTRFSPSFQG

SEQ ID NO: 280 - protein, 19 aa, synthetic construct
  REGION 1..19: note = Modified CDR
MGIINPVDSDTNYNPSFQG

SEQ ID NO: 281 - protein, 19 aa, synthetic construct
  REGION 1..19: note = Modified CDR
MGIINPVDSDTRFNPSFQG

SEQ ID NO: 282 - protein, 19 aa, synthetic construct
  REGION 1..19: note = Modified CDR
MGIINPVDSDTRYNPSFQG

SEQ ID NO: 283 - protein, 19 aa, synthetic construct
  REGION 1..19: note = Modified CDR
MGIINPVDSDTRYSPSFQG

SEQ ID NO: 284 - protein, 19 aa, synthetic construct
  REGION 1..19: note = Modified CDR
MGIINPVNGDTKFNPSFQG

SEQ ID NO: 285 - protein, 19 aa, synthetic construct
  REGION 1..19: note = Modified CDR
MGIINPVNGDTKYNPSFQG

SEQ ID NO: 286 - protein, 19 aa, synthetic construct
  REGION 1..19: note = Modified CDR
MGIINPVNGDTKYSPSFQG

SEQ ID NO: 287 - protein, 19 aa, synthetic construct
  REGION 1..19: note = Modified CDR
MGIINPVNGDTNFNPSFQG

SEQ ID NO: 288 - protein, 19 aa, synthetic construct
  REGION 1..19: note = Modified CDR
MGIINPVNGDTNFSPSFQG

SEQ ID NO: 289 - protein, 19 aa, synthetic construct
  REGION 1..19: note = Modified CDR
MGIINPVNGDTNYSPSFQG

SEQ ID NO: 290 - protein, 19 aa, synthetic construct
  REGION 1..19: note = Modified CDR
MGIINPVNGDTRFNPSFQG

SEQ ID NO: 291 - protein, 19 aa, synthetic construct
  REGION 1..19: note = Modified CDR
MGIINPVNGDTRFSPSFQG

SEQ ID NO: 292 - protein, 19 aa, synthetic construct
  REGION 1..19: note = Modified CDR
MGIINPVNGDTRYNPSFQG

SEQ ID NO: 293 - protein, 19 aa, synthetic construct
  REGION 1..19: note = Modified CDR
MGIINPVNGDTRYSPSFQG

SEQ ID NO: 294 - protein, 19 aa, synthetic construct
  REGION 1..19: note = Modified CDR
MGIINPVNSDTKYNPSFQG

SEQ ID NO: 295 - protein, 19 aa, synthetic construct
  REGION 1..19: note = Modified CDR
MGIINPVNSDTNFNPSFQG

SEQ ID NO: 296 - protein, 19 aa, synthetic construct
  REGION 1..19: note = Modified CDR
MGIINPVNSDTNYSPSFQG

SEQ ID NO: 297 - protein, 19 aa, synthetic construct
  REGION 1..19: note = Modified CDR
MGIINPVNSDTRFSPSFQG

SEQ ID NO: 298 - protein, 19 aa, synthetic construct
  REGION 1..19: note = Modified CDR
MGIINPVNSDTRYNPSFQG

SEQ ID NO: 299 - protein, 19 aa, synthetic construct
  REGION 1..19: note = Modified CDR
MGIINPVNSDTRYSPSFQG

SEQ ID NO: 300 - protein, 19 aa, synthetic construct
  REGION 1..19: note = Modified CDR
MGNINPVDGDTRYNPSFQG

SEQ ID NO: 301 - protein, 19 aa, synthetic construct
  REGION 1..19: note = Modified CDR
MGVINPVNSDTNYNPSFQG